European Patent Application EP 4 810 523 A1, published September 23, 2026. Title: 一种靶向C3b的双功能融合蛋白及其制备方法与用途. Applicant: 沈阳三生制药有限责任公司. The sequence listing filed with the application follows.

SEQUENCE LISTING (15 sequences)

SEQ ID NO: 1 - DNA, 357 bp, synthetic construct
  source 1..357: mol_type = other DNA; note = Nucleotide sequence of CRIg
ggccggcctatcctggaggtgcctgagtctgtgaccggcccttggaagggcgatgtgaacctgccttgcacctacgatcctctgcagggctacacccaggttctggtgaagtggctggtgcagaggggcagcgaccccgtgaccatctttctgcgcgactcctccggcgaccacatccagcaggccaagtaccagggcaggctgcacgtgtcccacaaggtgcccggcgacgtgtctctgcagctgtccaccctggagatggacgaccgctcccactatacctgcgaggtgacctggcagactcctgacggcaaccaggtggtgagagataagattaccgagctgagagtgcagaag

SEQ ID NO: 2 - protein, 119 aa, synthetic construct
  source 1..119: note = CRIg
GRPILEVPESVTGPWKGDVNLPCTYDPLQGYTQVLVKWLVQRGSDPVTIFLRDSSGDHIQQAKYQGRLHVSHKVPGDVSLQLSTLEMDDRSHYTCEVTWQTPDGNQVVRDKITELRVQK

SEQ ID NO: 3 - DNA, 915 bp, synthetic construct
  source 1..915: mol_type = other DNA; note = Nucleotide sequence of Factor H
gaggactgtaatgaactgcctcccagaagaaataccgaaatcctgaccggctcttggtctgatcagacctacccagaaggcacacaggctatctataaatgtagacctgggtatagaagtctgggcaatgtgatcatggtgtgtaggaagggagagtgggtggccctgaatcctctgagaaagtgccagaagaggccttgtggccatcccggcgataccccttttggtacttttacactgacaggcggcaatgtgtttgagtatggcgtgaaggccgtgtatacatgtaatgagggttatcagctgctgggcgagattaattatagagagtgtgatacagatggctggaccaatgatattcctatttgtgaagtggtgaagtgtctgcctgtgaccgcccccgagaatggaaagatcgtgagcagcgccatggagcccgatcgcgagtaccattttggccaggctgtgagattcgtgtgtaacagcggctacaagatcgaaggcgacgaggagatgcactgctctgatgacggcttttggtccaaggagaagccaaagtgcgtggagatctcctgcaagtctcctgacgtgatcaacggcagcccaatctctcagaagatcatctacaaggagaatgagaggttccagtacaagtgcaacatgggctacgagtactccgagagaggcgacgctgtgtgcaccgagtctggctggcggcctctgccaagctgcgaggagaagtcctgtgacaacccttatatcccaaacggcgactacagccctctgagaatcaagcataggacaggcgacgagatcacctaccagtgtaggaacggcttctaccccgctaccagaggcaacaccgccaagtgtacctccaccggctggatccctgccccccgatgcaccctgaag

SEQ ID NO: 4 - protein, 305 aa, synthetic construct
  source 1..305: note = Factor H
EDCNELPPRRNTEILTGSWSDQTYPEGTQAIYKCRPGYRSLGNVIMVCRKGEWVALNPLRKCQKRPCGHPGDTPFGTFTLTGGNVFEYGVKAVYTCNEGYQLLGEINYRECDTDGWTNDIPICEVVKCLPVTAPENGKIVSSAMEPDREYHFGQAVRFVCNSGYKIEGDEEMHCSDDGFWSKEKPKCVEISCKSPDVINGSPISQKIIYKENERFQYKCNMGYEYSERGDAVCTESGWRPLPSCEEKSCDNPYIPNGDYSPLRIKHRTGDEITYQCRNGFYPATRGNTAKCTSTGWIPAPRCTLK

SEQ ID NO: 5 - DNA, 672 bp, synthetic construct
  source 1..672: mol_type = other DNA; note = Nucleotide sequence of IgG4-Fc
cccccatgcccctcctgccctgcacctgagttcctgggcggcccttccgtgttcctgttccccccaaagcccaaggataccctgatgatcagccggacccctgaggtgacctgcgtggtggtggacgtgtcccaggaggaccccgaggtgcagttcaactggtacgtggacggcgtggaggtgcataacgccaagaccaagcccagagaggagcagtttaacagcacatacagagtggtgagcgtgctgacagtgctgcaccaggactggctgaatggcaaggagtacaagtgcaaggtgtctaataagggcctgcctagctctatcgaaaagaccatttctaaggctaagggccagcccagagagccacaggtgtacaccctgcccccttctcaggaggagatgaccaagaaccaggtgtctctgacctgcctggtgaagggcttttacccttctgatatcgccgtggagtgggagagcaacggacagcctgagaataattataagaccactccacctgtgctggatagcgatggcagcttcttcctgtactccagactgactgtggataagtctaggtggcaggagggcaatgtgttttcctgtagtgtgatgcatgaggccctgcataatcattatacccagaagtctctgtctctgtccctgggcaag

SEQ ID NO: 6 - protein, 224 aa, synthetic construct
  source 1..224: note = IgG4-Fc
PPCPSCPAPEFLGGPSVFLFPPKPKDTLMISRTPEVTCVVVDVSQEDPEVQFNWYVDGVEVHNAKTKPREEQFNSTYRVVSVLTVLHQDWLNGKEYKCKVSNKGLPSSIEKTISKAKGQPREPQVYTLPPSQEEMTKNQVSLTCLVKGFYPSDIAVEWESNGQPENNYKTTPPVLDSDGSFFLYSRLTVDKSRWQEGNVFSCSVMHEALHNHYTQKSLSLSLGK

SEQ ID NO: 7 - protein, 663 aa, synthetic construct
  source 1..663: note = CRIg-L-FH-FCG4
GRPILEVPESVTGPWKGDVNLPCTYDPLQGYTQVLVKWLVQRGSDPVTIFLRDSSGDHIQQAKYQGRLHVSHKVPGDVSLQLSTLEMDDRSHYTCEVTWQTPDGNQVVRDKITELRVQKSGGGGSGGGGSGGGGEDCNELPPRRNTEILTGSWSDQTYPEGTQAIYKCRPGYRSLGNVIMVCRKGEWVALNPLRKCQKRPCGHPGDTPFGTFTLTGGNVFEYGVKAVYTCNEGYQLLGEINYRECDTDGWTNDIPICEVVKCLPVTAPENGKIVSSAMEPDREYHFGQAVRFVCNSGYKIEGDEEMHCSDDGFWSKEKPKCVEISCKSPDVINGSPISQKIIYKENERFQYKCNMGYEYSERGDAVCTESGWRPLPSCEEKSCDNPYIPNGDYSPLRIKHRTGDEITYQCRNGFYPATRGNTAKCTSTGWIPAPRCTLKPPCPPCPAPEFLGGPSVFLFPPKPKDTLMISRTPEVTCVVVDVSQEDPEVQFNWYVDGVEVHNAKTKPREEQFNSTYRVVSVLTVLHQDWLNGKEYKCKVSNKGLPSSIEKTISKAKGQPREPQVYTLPPSQEEMTKNQVSLTCLVKGFYPSDIAVEWESNGQPENNYKTTPPVLDSDGSFFLYSRLTVDKSRWQEGNVFSCSVMHEALHNHYTQKSLSLSLGK

SEQ ID NO: 8 - protein, 663 aa, synthetic construct
  source 1..663: note = CRIg-L(GS)-FH-FCG4
GRPILEVPESVTGPWKGDVNLPCTYDPLQGYTQVLVKWLVQRGSDPVTIFLRDSSGDHIQQAKYQGRLHVSHKVPGDVSLQLSTLEMDDRSHYTCEVTWQTPDGNQVVRDKITELRVQKGGGGSGGGGSGGGGSEDCNELPPRRNTEILTGSWSDQTYPEGTQAIYKCRPGYRSLGNVIMVCRKGEWVALNPLRKCQKRPCGHPGDTPFGTFTLTGGNVFEYGVKAVYTCNEGYQLLGEINYRECDTDGWTNDIPICEVVKCLPVTAPENGKIVSSAMEPDREYHFGQAVRFVCNSGYKIEGDEEMHCSDDGFWSKEKPKCVEISCKSPDVINGSPISQKIIYKENERFQYKCNMGYEYSERGDAVCTESGWRPLPSCEEKSCDNPYIPNGDYSPLRIKHRTGDEITYQCRNGFYPATRGNTAKCTSTGWIPAPRCTLKPPCPPCPAPEFLGGPSVFLFPPKPKDTLMISRTPEVTCVVVDVSQEDPEVQFNWYVDGVEVHNAKTKPREEQFNSTYRVVSVLTVLHQDWLNGKEYKCKVSNKGLPSSIEKTISKAKGQPREPQVYTLPPSQEEMTKNQVSLTCLVKGFYPSDIAVEWESNGQPENNYKTTPPVLDSDGSFFLYSRLTVDKSRWQEGNVFSCSVMHEALHNHYTQKSLSLSLGK

SEQ ID NO: 9 - protein, 663 aa, synthetic construct
  source 1..663: note = CRIg-L(GS)-FH-FCG4-Q64R
GRPILEVPESVTGPWKGDVNLPCTYDPLQGYTQVLVKWLVQRGSDPVTIFLRDSSGDHIQQAKYRGRLHVSHKVPGDVSLQLSTLEMDDRSHYTCEVTWQTPDGNQVVRDKITELRVQKGGGGSGGGGSGGGGSEDCNELPPRRNTEILTGSWSDQTYPEGTQAIYKCRPGYRSLGNVIMVCRKGEWVALNPLRKCQKRPCGHPGDTPFGTFTLTGGNVFEYGVKAVYTCNEGYQLLGEINYRECDTDGWTNDIPICEVVKCLPVTAPENGKIVSSAMEPDREYHFGQAVRFVCNSGYKIEGDEEMHCSDDGFWSKEKPKCVEISCKSPDVINGSPISQKIIYKENERFQYKCNMGYEYSERGDAVCTESGWRPLPSCEEKSCDNPYIPNGDYSPLRIKHRTGDEITYQCRNGFYPATRGNTAKCTSTGWIPAPRCTLKPPCPPCPAPEFLGGPSVFLFPPKPKDTLMISRTPEVTCVVVDVSQEDPEVQFNWYVDGVEVHNAKTKPREEQFNSTYRVVSVLTVLHQDWLNGKEYKCKVSNKGLPSSIEKTISKAKGQPREPQVYTLPPSQEEMTKNQVSLTCLVKGFYPSDIAVEWESNGQPENNYKTTPPVLDSDGSFFLYSRLTVDKSRWQEGNVFSCSVMHEALHNHYTQKSLSLSLGK

SEQ ID NO: 10 - protein, 663 aa, synthetic construct
  source 1..663: note = CRIg-L(GS)-FH-FCG4-M86Y
GRPILEVPESVTGPWKGDVNLPCTYDPLQGYTQVLVKWLVQRGSDPVTIFLRDSSGDHIQQAKYQGRLHVSHKVPGDVSLQLSTLEYDDRSHYTCEVTWQTPDGNQVVRDKITELRVQKGGGGSGGGGSGGGGSEDCNELPPRRNTEILTGSWSDQTYPEGTQAIYKCRPGYRSLGNVIMVCRKGEWVALNPLRKCQKRPCGHPGDTPFGTFTLTGGNVFEYGVKAVYTCNEGYQLLGEINYRECDTDGWTNDIPICEVVKCLPVTAPENGKIVSSAMEPDREYHFGQAVRFVCNSGYKIEGDEEMHCSDDGFWSKEKPKCVEISCKSPDVINGSPISQKIIYKENERFQYKCNMGYEYSERGDAVCTESGWRPLPSCEEKSCDNPYIPNGDYSPLRIKHRTGDEITYQCRNGFYPATRGNTAKCTSTGWIPAPRCTLKPPCPPCPAPEFLGGPSVFLFPPKPKDTLMISRTPEVTCVVVDVSQEDPEVQFNWYVDGVEVHNAKTKPREEQFNSTYRVVSVLTVLHQDWLNGKEYKCKVSNKGLPSSIEKTISKAKGQPREPQVYTLPPSQEEMTKNQVSLTCLVKGFYPSDIAVEWESNGQPENNYKTTPPVLDSDGSFFLYSRLTVDKSRWQEGNVFSCSVMHEALHNHYTQKSLSLSLGK

SEQ ID NO: 11 - protein, 663 aa, synthetic construct
  source 1..663: note = CRIg-L(GS)-FH-FCG4-Q64R-M86Y
GRPILEVPESVTGPWKGDVNLPCTYDPLQGYTQVLVKWLVQRGSDPVTIFLRDSSGDHIQQAKYRGRLHVSHKVPGDVSLQLSTLEYDDRSHYTCEVTWQTPDGNQVVRDKITELRVQKGGGGSGGGGSGGGGSEDCNELPPRRNTEILTGSWSDQTYPEGTQAIYKCRPGYRSLGNVIMVCRKGEWVALNPLRKCQKRPCGHPGDTPFGTFTLTGGNVFEYGVKAVYTCNEGYQLLGEINYRECDTDGWTNDIPICEVVKCLPVTAPENGKIVSSAMEPDREYHFGQAVRFVCNSGYKIEGDEEMHCSDDGFWSKEKPKCVEISCKSPDVINGSPISQKIIYKENERFQYKCNMGYEYSERGDAVCTESGWRPLPSCEEKSCDNPYIPNGDYSPLRIKHRTGDEITYQCRNGFYPATRGNTAKCTSTGWIPAPRCTLKPPCPPCPAPEFLGGPSVFLFPPKPKDTLMISRTPEVTCVVVDVSQEDPEVQFNWYVDGVEVHNAKTKPREEQFNSTYRVVSVLTVLHQDWLNGKEYKCKVSNKGLPSSIEKTISKAKGQPREPQVYTLPPSQEEMTKNQVSLTCLVKGFYPSDIAVEWESNGQPENNYKTTPPVLDSDGSFFLYSRLTVDKSRWQEGNVFSCSVMHEALHNHYTQKSLSLSLGK

SEQ ID NO: 12 - protein, 648 aa, synthetic construct
  source 1..648: note = CRIg-FH-FCG4-Q64R
GRPILEVPESVTGPWKGDVNLPCTYDPLQGYTQVLVKWLVQRGSDPVTIFLRDSSGDHIQQAKYRGRLHVSHKVPGDVSLQLSTLEMDDRSHYTCEVTWQTPDGNQVVRDKITELRVQKEDCNELPPRRNTEILTGSWSDQTYPEGTQAIYKCRPGYRSLGNVIMVCRKGEWVALNPLRKCQKRPCGHPGDTPFGTFTLTGGNVFEYGVKAVYTCNEGYQLLGEINYRECDTDGWTNDIPICEVVKCLPVTAPENGKIVSSAMEPDREYHFGQAVRFVCNSGYKIEGDEEMHCSDDGFWSKEKPKCVEISCKSPDVINGSPISQKIIYKENERFQYKCNMGYEYSERGDAVCTESGWRPLPSCEEKSCDNPYIPNGDYSPLRIKHRTGDEITYQCRNGFYPATRGNTAKCTSTGWIPAPRCTLKPPCPPCPAPEFLGGPSVFLFPPKPKDTLMISRTPEVTCVVVDVSQEDPEVQFNWYVDGVEVHNAKTKPREEQFNSTYRVVSVLTVLHQDWLNGKEYKCKVSNKGLPSSIEKTISKAKGQPREPQVYTLPPSQEEMTKNQVSLTCLVKGFYPSDIAVEWESNGQPENNYKTTPPVLDSDGSFFLYSRLTVDKSRWQEGNVFSCSVMHEALHNHYTQKSLSLSLGK

SEQ ID NO: 13 - protein, 648 aa, synthetic construct
  source 1..648: note = CRIg -FH-FCG4-M86Y
GRPILEVPESVTGPWKGDVNLPCTYDPLQGYTQVLVKWLVQRGSDPVTIFLRDSSGDHIQQAKYQGRLHVSHKVPGDVSLQLSTLEYDDRSHYTCEVTWQTPDGNQVVRDKITELRVQKEDCNELPPRRNTEILTGSWSDQTYPEGTQAIYKCRPGYRSLGNVIMVCRKGEWVALNPLRKCQKRPCGHPGDTPFGTFTLTGGNVFEYGVKAVYTCNEGYQLLGEINYRECDTDGWTNDIPICEVVKCLPVTAPENGKIVSSAMEPDREYHFGQAVRFVCNSGYKIEGDEEMHCSDDGFWSKEKPKCVEISCKSPDVINGSPISQKIIYKENERFQYKCNMGYEYSERGDAVCTESGWRPLPSCEEKSCDNPYIPNGDYSPLRIKHRTGDEITYQCRNGFYPATRGNTAKCTSTGWIPAPRCTLKPPCPPCPAPEFLGGPSVFLFPPKPKDTLMISRTPEVTCVVVDVSQEDPEVQFNWYVDGVEVHNAKTKPREEQFNSTYRVVSVLTVLHQDWLNGKEYKCKVSNKGLPSSIEKTISKAKGQPREPQVYTLPPSQEEMTKNQVSLTCLVKGFYPSDIAVEWESNGQPENNYKTTPPVLDSDGSFFLYSRLTVDKSRWQEGNVFSCSVMHEALHNHYTQKSLSLSLGK

SEQ ID NO: 14 - protein, 648 aa, synthetic construct
  source 1..648: note = CRIg-FH-FCG4-Q64R-M86Y
GRPILEVPESVTGPWKGDVNLPCTYDPLQGYTQVLVKWLVQRGSDPVTIFLRDSSGDHIQQAKYRGRLHVSHKVPGDVSLQLSTLEYDDRSHYTCEVTWQTPDGNQVVRDKITELRVQKEDCNELPPRRNTEILTGSWSDQTYPEGTQAIYKCRPGYRSLGNVIMVCRKGEWVALNPLRKCQKRPCGHPGDTPFGTFTLTGGNVFEYGVKAVYTCNEGYQLLGEINYRECDTDGWTNDIPICEVVKCLPVTAPENGKIVSSAMEPDREYHFGQAVRFVCNSGYKIEGDEEMHCSDDGFWSKEKPKCVEISCKSPDVINGSPISQKIIYKENERFQYKCNMGYEYSERGDAVCTESGWRPLPSCEEKSCDNPYIPNGDYSPLRIKHRTGDEITYQCRNGFYPATRGNTAKCTSTGWIPAPRCTLKPPCPPCPAPEFLGGPSVFLFPPKPKDTLMISRTPEVTCVVVDVSQEDPEVQFNWYVDGVEVHNAKTKPREEQFNSTYRVVSVLTVLHQDWLNGKEYKCKVSNKGLPSSIEKTISKAKGQPREPQVYTLPPSQEEMTKNQVSLTCLVKGFYPSDIAVEWESNGQPENNYKTTPPVLDSDGSFFLYSRLTVDKSRWQEGNVFSCSVMHEALHNHYTQKSLSLSLGK

SEQ ID NO: 15 - protein, 663 aa, synthetic construct
  source 1..663: note = CRIg-L(GS)-FH-FCG4-YTE -M86Y
GRPILEVPESVTGPWKGDVNLPCTYDPLQGYTQVLVKWLVQRGSDPVTIFLRDSSGDHIQQAKYQGRLHVSHKVPGDVSLQLSTLEYDDRSHYTCEVTWQTPDGNQVVRDKITELRVQKGGGGSGGGGSGGGGSEDCNELPPRRNTEILTGSWSDQTYPEGTQAIYKCRPGYRSLGNVIMVCRKGEWVALNPLRKCQKRPCGHPGDTPFGTFTLTGGNVFEYGVKAVYTCNEGYQLLGEINYRECDTDGWTNDIPICEVVKCLPVTAPENGKIVSSAMEPDREYHFGQAVRFVCNSGYKIEGDEEMHCSDDGFWSKEKPKCVEISCKSPDVINGSPISQKIIYKENERFQYKCNMGYEYSERGDAVCTESGWRPLPSCEEKSCDNPYIPNGDYSPLRIKHRTGDEITYQCRNGFYPATRGNTAKCTSTGWIPAPRCTLKPPCPPCPAPEFLGGPSVFLFPPKPKDTLYITREPEVTCVVVDVSQEDPEVQFNWYVDGVEVHNAKTKPREEQFNSTYRVVSVLTVLHQDWLNGKEYKCKVSNKGLPSSIEKTISKAKGQPREPQVYTLPPSQEEMTKNQVSLTCLVKGFYPSDIAVEWESNGQPENNYKTTPPVLDSDGSFFLYSRLTVDKSRWQEGNVFSCSVMHEALHNHYTQKSLSLSLGK